European Patent Specification EP 3 727 332 B1, published March 12, 2025. Title: Liquid pharmaceutical composition. Applicant: Sanofi. The sequence listing filed with the application follows.

SEQUENCE LISTING (2 sequences)

SEQ ID NO: 1 - protein, 31 aa, Artificial Sequence
  Liraglutide
  MOD_RES (20)..(20): Lys is functionalized at the amino side chain group as Lys((S)-4-carboxy-4-hexadecanoylamino-butyryl)
HAEGTFTSDVSSYLEGQAAKEFIAWLVRGRG

SEQ ID NO: 2 - protein, 39 aa, Artificial Sequence
  Exendin-4 analogue
  MOD_RES (2)..(2): Xaa is a D-Ser
  MOD_RES (14)..(14): Lys is functionalized at the amino side chain group as Lys((S)-4-carboxy-4-hexadecanoylamino-butyryl)
  MOD_RES (39)..(39): Ser is modified with an NH2 group
HXQGTFTSDLSKQKESKAAQDFIEWLKAGGPSSGAPPPS